European Patent Specification EP 4 409 027 B1, published November 19, 2025. Title: TEMPERATURE-SELECTABLE FRET CASSETTE SIGNALING. Applicant: Gen-Probe Incorporated. The sequence listing filed with the application follows.

SEQUENCE LISTING (16 sequences)

SEQ ID NO: 1 - skipped

SEQ ID NO: 2 - DNA, 31 bp, synthetic construct
  source 1..31: mol_type = other DNA
  misc_feature 14..31: function = Complementary to positions 22-39 of SEQ ID NO:3 (Target strand nucleic acid)
  misc_feature 31: function = 3'-hexanediol
acgggacgcggagnnnnnnnnnnnnnnnnnn

SEQ ID NO: 3 - skipped

SEQ ID NO: 4 - DNA, 14 bp, synthetic construct
  source 1..14: mol_type = other DNA
  misc_feature 1..13: function = Complementary to positions 27-39 of SEQ ID NO:5 (FRET cassette)
acgggacgcggagn

SEQ ID NO: 5 - DNA, 39 bp, synthetic construct
  source 1..39: mol_type = other DNA
  misc_feature 1: function = 5' HEX fluorophore
  misc_feature 3..4: function = Quencher moiety joined to oligo between base positions 3 and 4
  misc_feature 4..11: function = Complementary to positions 16-23 in a hairpin configuration
  misc_feature 39: function = 3'-hexanediol
tctnnnnnnnnttttnnnnnnnnagactccgcgtcccgt

SEQ ID NO: 6 - DNA, 38 bp, synthetic construct
  source 1..38: mol_type = other DNA
  misc_feature 2..3: function = Quencher moiety joined to oligo between base positions 2 and 3
  misc_feature 3..10: function = Complementary to positions 15-22 in a hairpin configuration
  misc_feature 38: function = 3'-hexanediol
ctnnnnnnnnttttnnnnnnnnagactccgcgtcccgt

SEQ ID NO: 7 - DNA, 46 bp, synthetic construct
  source 1..46: mol_type = other DNA
  misc_feature 10: function = HEX fluorophore joined to oligonucleotide at position 10
  misc_feature 13..14: function = Quencher moiety joined to oligo between base positions 13 and 14
  misc_feature 14..21: function = Complementary to positions 26-33 in a hairpin configuration
  misc_feature 37..46: function = Complementary to positions 1-10 of SEQ ID NO:8 (cleaved flap from primary probe)
  misc_feature 46: function = 3'-hexanediol
caactgtatgtctnnnnnnnnttttnnnnnnnnagacctcggcgcg

SEQ ID NO: 8 - DNA, 11 bp, synthetic construct
  source 1..11: mol_type = other DNA
  misc_feature 1..10: function = Complementary to positions 37-46 of SEQ ID NO:7 (5' flap FRET cassette)
cgcgccgaggn

SEQ ID NO: 9 - DNA, 11 bp, synthetic construct
  source 1..11: mol_type = other DNA
  misc_feature 10: function = Position 10 modified with HEX fluorophore
caactgtatgt

SEQ ID NO: 10 - DNA, 10 bp, synthetic construct
  source 1..10: mol_type = other DNA
  misc_feature 1: function = 5' quencher moiety
catacagttg

SEQ ID NO: 11 - DNA, 34 bp, synthetic construct
  source 1..34: mol_type = other DNA
  misc_feature 1: function = 5' HEX fluorophore
  misc_feature 3..4: function = Quencher moiety joined to oligo between base positions 3 and 4
  misc_feature 4..9: function = complementary to positions 14-19 in a hairpin configuration
  misc_feature 23..34: function = Complementary to positions 1-12 of SEQ ID NO:12 (cleaved flap from Target 1)
  misc_feature 34: function = 3'-hexanediol
tctnnnnnnttttnnnnnnagacgtccgtggcct

SEQ ID NO: 12 - DNA, 13 bp, synthetic construct
  source 1..13: mol_type = other DNA
  misc_feature 1..12: function = Complementary to positions 23-34 of SEQ ID NO:11 (flapless FRET cassette)
aggccacggacgn

SEQ ID NO: 13 - DNA, 48 bp, synthetic construct
  source 1..48: mol_type = other DNA
  misc_feature 10: function = Position 10 modified with HEX fluorophore
  misc_feature 13..14: function = Quencher moiety joined to oligo beetween base positions 13-14
  misc_feature 14..21: function = Complementary to positions 26-33 in a hairpin configuration
  misc_feature 37..48: function = Complementary to positions 1-12 of SEQ ID NO:14 (cleaved flap from Target 3 primary probe)
  misc_feature 48: function = 3'-hexanediol
cagctgcatgtctnnnnnnnnttttnnnnnnnnagactccgcgtccgt

SEQ ID NO: 14 - DNA, 13 bp, synthetic construct
  source 1..13: mol_type = other DNA
  misc_feature 1..12: function = Complementary to positions 37-48 of SEQ ID NO:13 (5' flap FRET cassette 2)
acggacgcggagn

SEQ ID NO: 15 - DNA, 11 bp, synthetic construct
  source 1..11: mol_type = other DNA
  misc_feature 1..10: function = Complementary to positions 1-10 of SEQ ID NO:16 (masking oligo 2)
  misc_feature 10: function = Position 10 modified with HEX fluorophore
cagctgcatgt

SEQ ID NO: 16 - DNA, 10 bp, synthetic construct
  source 1..10: mol_type = other DNA
  misc_feature 1..10: function = Complementary to positions 1-10 of SEQ ID NO:15 (cassette cleaved flap 2)
  misc_feature 1: function = 5' quencher moiety
catgcagctg